European Patent Application EP 4 674 966 A1, published January 7, 2026. Title: Target protein degradation method. Applicant: 大学共同利用機関法人情報・システム研究機構. The sequence listing filed with the application follows.

SEQUENCE LISTING (17 sequences)

SEQ ID NO: 1 - DNA, 1728 bp, Oryza sativa
  source 1..1728: mol_type = other DNA
atgacgtacttcccggaggaggtggtggagcacatcttcagcttcctgccggcgcagcgcgaccgcaacacggtctcgctcgtctgcaaggtgtggtacgagatcgagaggctgagccgccgcggcgtcttcgtgggcaactgctacgccgtgcgcgccggccgcgtcgccgcgcggttccccaacgtgcgggcgctcacggtgaaggggaagccccacttcgccgacttcaacctcgtgccccccgactggggcggctacgcggggccgtggatcgaggcggccgcgaggggatgccacggcctggaggagctcaggatgaagcggatggtggtgtccgacgagagcctcgagctgctggctcgctcgttcccgcggttcagggctcttgttcttatcagctgcgaggggttcagcactgacgggctagccgccgtcgcgagccattgcaagcttctgagggagttggatttgcaggaaaatgaagtggaggatcgagggcctaggtggctttcctgcttccctgattcctgcacatcacttgtctcattgaattttgcctgcatcaaaggggaggttaatgctggttcactggagagacttgttagcaggtccccaaacctgcggagtttgaggctgaatcgatctgtatcggtagatacacttgcaaagatactactgcgtacccctaacttggaggatttggggacagggaatttgacagatgacttccaaactgagtcctactttaagcttaccagtgctctggagaaatgcaagatgttgaggagtttgtctggattctgggatgcttctcctgtttgcctgtcatttatctaccccctgtgtgctcaactgacaggattgaacttgagctatgcccccacacttgatgcttctgaccttacaaaaatgattagccgctgtgtgaagctccaacgcctttgggtactggattgtatctcggacaaaggcttgcaagtggtggcctccagttgcaaagacttgcaagaactcagggtatttccatcagatttctacgtagctggttattctgcagtgacagaggagggacttgttgcagtatccttgggctgtccaaaactgaactcactactgtacttctgtcaccaaatgactaatgctgcactagttactgtcgccaagaactgtccaaatttcacacgattcagactttgtattcttgagccagggaagcctgatgttgtgacaagccaaccattagatgaaggctttggagctattgttcgtgagtgcaagggattacaacgtttgtcaatatctggtcttctcacagacaaagttttcatgtatattgggaaatatgcaaaacaacttgagatgctttctatagcatttgctggtgacagtgataagggtatgatgcatgttatgaatggatgcaagaatttaaggaaactggagataagagatagcccgtttggtgatgctgcactcttggggaattttgctaggtacgagacaatgcgatccctttggatgtcatcttgcaatgtcacgttaaaggggtgccaagtccttgcgtcaaagatgccgatgctcaatgttgaggtcataaatgagcgggatggtagcaatgaaatggaggaaaaccatggagatctgcctaaagtggagaaattatatgtgtaccgcacaactgctggggcgagggatgatgcaccaaattttgttaaaatcctatag

SEQ ID NO: 2 - DNA, 1728 bp, synthetic construct
  misc_feature 1..1728: note = OsTIR1 DNA optimized for human codon
  source 1..1728: mol_type = other DNA
atgacatactttcctgaagaggtcgtcgaacacatttttagcttcctgcctgcacagagagatagaaacacagtgagcctggtctgcaaagtgtggtacgagatcgaacgcctgagccggagaggagtgttcgtcggcaactgctatgctgtgagagcaggcagggtcgccgctaggtttccaaatgtgcgcgcactgaccgtcaaggggaaaccccacttcgccgactttaacctggtgccccctgattggggaggatacgccggcccttggatcgaggcagccgctcgcggctgtcatggactggaggaactgcgcatgaagcgaatggtggtctctgacgaaagtctggagctgctggctcggagcttccctaggtttcgcgcactggtgctgatttcttgcgaaggcttcagcaccgatggactggcagccgtggcctcccactgtaagctgctgcgggagctggacctccaggagaatgaagtggaggatagaggccccagatggctgtcttgcttcccagactcatgtaccagcctggtgtccctgaactttgcctgcatcaaaggcgaagtgaatgctgggtccctggagcggctggtctcaagaagccccaacctgaggtctctgcggctgaaccggagcgtgagcgtggacactctggctaagattctgctgagaacccctaacctggaggatctgggaaccggcaatctgacagacgatttccagacagaatcctactttaaactgacttctgccctggagaagtgtaaaatgctgaggagtctgtcaggattctgggatgcttcacccgtgtgcctgagctttatctaccctctgtgtgcacagctgacaggcctgaacctgagctatgcaccaaccctggacgccagtgatctgacaaagatgatctcacgctgcgtgaaactccagcgactgtgggtgctggactgtatttccgataaggggctccaggtggtcgccagctcctgcaaggacctccaggagctgagagtgttcccatctgatttttacgtggccggatatagtgctgtcactgaggaaggcctggtggcagtctcactgggatgcccaaagctgaacagcctgctgtatttctgtcatcagatgactaatgctgcactggtgaccgtcgccaagaactgccctaatttcacccgatttcggctgtgtattctggaaccaggcaaacccgacgtggtcacatcccagccactggatgaagggtttggagctatcgtgagagagtgcaagggactccagaggctgagcatttccggcctgctgacagacaaagtgttcatgtacatcggcaagtatgctaagcagctggagatgctgagcattgcatttgccggagactccgataagggcatgatgcacgtgatgaacgggtgtaagaatctgcgaaaactggaaatccgggacagccctttcggggatgccgctctgctgggaaactttgccagatacgagacaatgaggagcctgtggatgtctagttgcaatgtgactctgaagggctgtcaggtcctggctagtaaaatgcctatgctgaacgtggaagtcattaatgagcgggacgggtctaacgaaatggaggaaaatcatggcgacctgccaaaggtggagaaactgtatgtgtatcggaccaccgcaggggcaagagatgatgctcccaactttgtgaagattctgtga

SEQ ID NO: 3 - protein, 575 aa, Oryza sativa
MTYFPEEVVEHIFSFLPAQRDRNTVSLVCKVWYEIERLSRRGVFVGNCYAVRAGRVAARFPNVRALTVKGKPHFADFNLVPPDWGGYAGPWIEAAARGCHGLEELRMKRMVVSDESLELLARSFPRFRALVLISCEGFSTDGLAAVASHCKLLRELDLQENEVEDRGPRWLSCFPDSCTSLVSLNFACIKGEVNAGSLERLVSRSPNLRSLRLNRSVSVDTLAKILLRTPNLEDLGTGNLTDDFQTESYFKLTSALEKCKMLRSLSGFWDASPVCLSFIYPLCAQLTGLNLSYAPTLDASDLTKMISRCVKLQRLWVLDCISDKGLQVVASSCKDLQELRVFPSDFYVAGYSAVTEEGLVAVSLGCPKLNSLLYFCHQMTNAALVTVAKNCPNFTRFRLCILEPGKPDVVTSQPLDEGFGAIVRECKGLQRLSISGLLTDKVFMYIGKYAKQLEMLSIAFAGDSDKGMMHVMNGCKNLRKLEIRDSPFGDAALLGNFARYETMRSLWMSSCNVTLKGCQVLASKMPMLNVEVINERDGSNEMEENHGDLPKVEKLYVYRTTAGARDDAPNFVKIL

SEQ ID NO: 4 - protein, 575 aa, synthetic construct
  REGION 1..575: note = OsTIR1 F74A Protein
MTYFPEEVVEHIFSFLPAQRDRNTVSLVCKVWYEIERLSRRGVFVGNCYAVRAGRVAARFPNVRALTVKGKPHAADFNLVPPDWGGYAGPWIEAAARGCHGLEELRMKRMVVSDESLELLARSFPRFRALVLISCEGFSTDGLAAVASHCKLLRELDLQENEVEDRGPRWLSCFPDSCTSLVSLNFACIKGEVNAGSLERLVSRSPNLRSLRLNRSVSVDTLAKILLRTPNLEDLGTGNLTDDFQTESYFKLTSALEKCKMLRSLSGFWDASPVCLSFIYPLCAQLTGLNLSYAPTLDASDLTKMISRCVKLQRLWVLDCISDKGLQVVASSCKDLQELRVFPSDFYVAGYSAVTEEGLVAVSLGCPKLNSLLYFCHQMTNAALVTVAKNCPNFTRFRLCILEPGKPDVVTSQPLDEGFGAIVRECKGLQRLSISGLLTDKVFMYIGKYAKQLEMLSIAFAGDSDKGMMHVMNGCKNLRKLEIRDSPFGDAALLGNFARYETMRSLWMSSCNVTLKGCQVLASKMPMLNVEVINERDGSNEMEENHGDLPKVEKLYVYRTTAGARDDAPNFVKIL

SEQ ID NO: 5 - DNA, 1728 bp, synthetic construct
  misc_feature 1..1728: note = OsTIR1 F74A DNA
  source 1..1728: mol_type = other DNA
atgacatactttcctgaagaggtcgtcgaacacatttttagcttcctgcctgcacagagagatagaaacacagtgagcctggtctgcaaagtgtggtacgagatcgaacgcctgagccggagaggagtgttcgtcggcaactgctatgctgtgagagcaggcagggtcgccgctaggtttccaaatgtgcgcgcactgaccgtcaaggggaaaccccacgccgccgactttaacctggtgccccctgattggggaggatacgccggcccttggatcgaggcagccgctcgcggctgtcatggactggaggaactgcgcatgaagcgaatggtggtctctgacgaaagtctggagctgctggctcggagcttccctaggtttcgcgcactggtgctgatttcttgcgaaggcttcagcaccgatggactggcagccgtggcctcccactgtaagctgctgcgggagctggacctccaggagaatgaagtggaggatagaggccccagatggctgtcttgcttcccagactcatgtaccagcctggtgtccctgaactttgcctgcatcaaaggcgaagtgaatgctgggtccctggagcggctggtctcaagaagccccaacctgaggtctctgcggctgaaccggagcgtgagcgtggacactctggctaagattctgctgagaacccctaacctggaggatctgggaaccggcaatctgacagacgatttccagacagaatcctactttaaactgacttctgccctggagaagtgtaaaatgctgaggagtctgtcaggattctgggatgcttcacccgtgtgcctgagctttatctaccctctgtgtgcacagctgacaggcctgaacctgagctatgcaccaaccctggacgccagtgatctgacaaagatgatctcacgctgcgtgaaactccagcgactgtgggtgctggactgtatttccgataaggggctccaggtggtcgccagctcctgcaaggacctccaggagctgagagtgttcccatctgatttttacgtggccggatatagtgctgtcactgaggaaggcctggtggcagtctcactgggatgcccaaagctgaacagcctgctgtatttctgtcatcagatgactaatgctgcactggtgaccgtcgccaagaactgccctaatttcacccgatttcggctgtgtattctggaaccaggcaaacccgacgtggtcacatcccagccactggatgaagggtttggagctatcgtgagagagtgcaagggactccagaggctgagcatttccggcctgctgacagacaaagtgttcatgtacatcggcaagtatgctaagcagctggagatgctgagcattgcatttgccggagactccgataagggcatgatgcacgtgatgaacgggtgtaagaatctgcgaaaactggaaatccgggacagccctttcggggatgccgctctgctgggaaactttgccagatacgagacaatgaggagcctgtggatgtctagttgcaatgtgactctgaagggctgtcaggtcctggctagtaaaatgcctatgctgaacgtggaagtcattaatgagcgggacgggtctaacgaaatggaggaaaatcatggcgacctgccaaaggtggagaaactgtatgtgtatcggaccaccgcaggggcaagagatgatgctcccaactttgtgaagattctgtga

SEQ ID NO: 6 - protein, 575 aa, synthetic construct
  REGION 1..575: note = OsTIR1 F74G Protein
MTYFPEEVVEHIFSFLPAQRDRNTVSLVCKVWYEIERLSRRGVFVGNCYAVRAGRVAARFPNVRALTVKGKPHGADFNLVPPDWGGYAGPWIEAAARGCHGLEELRMKRMVVSDESLELLARSFPRFRALVLISCEGFSTDGLAAVASHCKLLRELDLQENEVEDRGPRWLSCFPDSCTSLVSLNFACIKGEVNAGSLERLVSRSPNLRSLRLNRSVSVDTLAKILLRTPNLEDLGTGNLTDDFQTESYFKLTSALEKCKMLRSLSGFWDASPVCLSFIYPLCAQLTGLNLSYAPTLDASDLTKMISRCVKLQRLWVLDCISDKGLQVVASSCKDLQELRVFPSDFYVAGYSAVTEEGLVAVSLGCPKLNSLLYFCHQMTNAALVTVAKNCPNFTRFRLCILEPGKPDVVTSQPLDEGFGAIVRECKGLQRLSISGLLTDKVFMYIGKYAKQLEMLSIAFAGDSDKGMMHVMNGCKNLRKLEIRDSPFGDAALLGNFARYETMRSLWMSSCNVTLKGCQVLASKMPMLNVEVINERDGSNEMEENHGDLPKVEKLYVYRTTAGARDDAPNFVKIL

SEQ ID NO: 7 - DNA, 1728 bp, synthetic construct
  misc_feature 1..1728: note = OsTIR1 F74G DNA
  source 1..1728: mol_type = other DNA
atgacatactttcctgaagaggtcgtcgaacacatttttagcttcctgcctgcacagagagatagaaacacagtgagcctggtctgcaaagtgtggtacgagatcgaacgcctgagccggagaggagtgttcgtcggcaactgctatgctgtgagagcaggcagggtcgccgctaggtttccaaatgtgcgcgcactgaccgtcaaggggaaaccccacggcgccgactttaacctggtgccccctgattggggaggatacgccggcccttggatcgaggcagccgctcgcggctgtcatggactggaggaactgcgcatgaagcgaatggtggtctctgacgaaagtctggagctgctggctcggagcttccctaggtttcgcgcactggtgctgatttcttgcgaaggcttcagcaccgatggactggcagccgtggcctcccactgtaagctgctgcgggagctggacctccaggagaatgaagtggaggatagaggccccagatggctgtcttgcttcccagactcatgtaccagcctggtgtccctgaactttgcctgcatcaaaggcgaagtgaatgctgggtccctggagcggctggtctcaagaagccccaacctgaggtctctgcggctgaaccggagcgtgagcgtggacactctggctaagattctgctgagaacccctaacctggaggatctgggaaccggcaatctgacagacgatttccagacagaatcctactttaaactgacttctgccctggagaagtgtaaaatgctgaggagtctgtcaggattctgggatgcttcacccgtgtgcctgagctttatctaccctctgtgtgcacagctgacaggcctgaacctgagctatgcaccaaccctggacgccagtgatctgacaaagatgatctcacgctgcgtgaaactccagcgactgtgggtgctggactgtatttccgataaggggctccaggtggtcgccagctcctgcaaggacctccaggagctgagagtgttcccatctgatttttacgtggccggatatagtgctgtcactgaggaaggcctggtggcagtctcactgggatgcccaaagctgaacagcctgctgtatttctgtcatcagatgactaatgctgcactggtgaccgtcgccaagaactgccctaatttcacccgatttcggctgtgtattctggaaccaggcaaacccgacgtggtcacatcccagccactggatgaagggtttggagctatcgtgagagagtgcaagggactccagaggctgagcatttccggcctgctgacagacaaagtgttcatgtacatcggcaagtatgctaagcagctggagatgctgagcattgcatttgccggagactccgataagggcatgatgcacgtgatgaacgggtgtaagaatctgcgaaaactggaaatccgggacagccctttcggggatgccgctctgctgggaaactttgccagatacgagacaatgaggagcctgtggatgtctagttgcaatgtgactctgaagggctgtcaggtcctggctagtaaaatgcctatgctgaacgtggaagtcattaatgagcgggacgggtctaacgaaatggaggaaaatcatggcgacctgccaaaggtggagaaactgtatgtgtatcggaccaccgcaggggcaagagatgatgctcccaactttgtgaagattctgtga

SEQ ID NO: 8 - protein, 64 aa, synthetic construct
  REGION 1..64: note = Mini auxin inducible degron
ACPKDPAKPPAKAQVVGWPPVRSYRKNVMVSCQKSSGGPEAAAFVKVSMDGAPYLRKIDLRMYK

SEQ ID NO: 9 - DNA, 345 bp, synthetic construct
  source 1..345: mol_type = other DNA
caagtccaactggtggagtctggtggcgctttggtgcagccaggtggctctctgcgtttgtcctgtgccgcttctggcttcccagtgaaccgctattccatgcgctggtatcgccaggctccaggcaaagagcgtgagtgggtagccggtatgtccagcgcgggtgatcgtagctcctatgaagactccgtgaagggccgtttcaccatcagccgtgacgatgcccgtaacacggtgtatctgcaaatgaacagcttgaaacctgaagatacggccgtgtattactgtaatgtgaacgtgggcttcgagtattggggccaaggcacccaggtcaccgtctccagc

SEQ ID NO: 10 - DNA, 345 bp, synthetic construct
  source 1..345: mol_type = other DNA
caagtccaactggtggagtctggtggcgctttggtgcagccaggtggctctctgcgtttgtcctgtgccgcttctggcttcccagtgaaccgctattccatgcgctggtatcgccaggctccaggccgcgagcgtgagtgggtagccggtatgtccagcgcgggtgatcgtagctcctatgaagactccgtgcggggccgtttcaccatcagccgtgacgatgcccgtaacacggtgtatctgcaaatgaacagcttgcgtcctgaagatacggccgtgtattactgtaatgtgaacgtgggcttcgagtattggggccaaggcacccaggtcaccgtctccagc

SEQ ID NO: 11 - DNA, 375 bp, synthetic construct
  source 1..375: mol_type = other DNA
caggttcaactgcaggaaagcgggggaggcttggttcaagccggagggagtctccggctctcatgtgctgcaagtgaacggaccttttctacttacgcaatggggtggtttcgccaggctccaggcagagaaagggagtttctggcacaaataaattggtccggtacaaccacctactatgccgaatcagtaaaagatcgaaccactatatcaagagataatgcaaaaaatactgtctacctggagatgaacaatcttaatgctgatgacacagggatttatttctgtgctgctcacccgcagcggggatggggttctactctggggtggacttactggggtcaggggacccaggtaactgtttcaagcacataa

SEQ ID NO: 12 - DNA, 375 bp, synthetic construct
  source 1..375: mol_type = other DNA
caggttcaactgcaggaaagcgggggaggcttggttcaagccggagggagtctccggctctcatgtgctgcaagtgaacggaccttttctacttacgcaatggggtggtttcgccaggctccaggcagagaaagggagtttctggcacaaataaattggtccggtacaaccacctactatgccgaatcagtacgcgatcgaaccactatatcaagagataatgcacgcaatactgtctacctggagatgaacaatcttaatgctgatgacacagggatttatttctgtgctgctcacccgcagcggggatggggttctactctggggtggacttactggggtcaggggacccaggtaactgtttcaagcacataa

SEQ ID NO: 13 - protein, 64 aa, synthetic construct
ACPRDPARPPARAQVVGWPPVRSYRRNVMVSCQRSSGGPEAAAFVRVSMDGAPYLRRIDLRMYR

SEQ ID NO: 14 - DNA, 294 bp, synthetic construct
  source 1..294: mol_type = other DNA
atgggctctgtatcttcagtccctacaaagctggaagtagtagcggcaacaccgacgagcctcctcatttcctgggacgcaccggcggtcaccgtcgattactatgttatcacttacggtgaaactggtggaaacagccccgttcagaaatttgaggttcctggaagcaaaagcactgccaccatttcaggtcttaaaccgggagtggactacacgataacggtctatgcttggggttggcacggccaagtgtattactatatgggctcacccatcagcatcaattatcgaacg

SEQ ID NO: 15 - protein, 98 aa, synthetic construct
MGSVSSVPTKLEVVAATPTSLLISWDAPAVTVDYYVITYGETGGNSPVQKFEVPGSKSTATISGLKPGVDYTITVYAWGWHGQVYYYMGSPISINYRT

SEQ ID NO: 16 - DNA, 294 bp, synthetic construct
  source 1..294: mol_type = other DNA
atgggctctgtatcttcagtccctacacggctggaagtagtagcggcaacaccgacgagcctcctcatttcctgggacgcaccggcggtcaccgtcgattactatgttatcacttacggtgaaactggtggaaacagccccgttcagcgctttgaggttcctggaagccgcagcactgccaccatttcaggtcttcgcccgggagtggactacacgataacggtctatgcttggggttggcacggccaagtgtattactatatgggctcacccatcagcatcaattatcgaacg

SEQ ID NO: 17 - protein, 98 aa, synthetic construct
MGSVSSVPTRLEVVAATPTSLLISWDAPAVTVDYYVITYGETGGNSPVQRFEVPGSRSTATISGLRPGVDYTITVYAWGWHGQVYYYMGSPISINYRT